European Patent Application EP 4 279 506 A1, published November 22, 2023. Title: B7-H3 CHIMERIC ANTIGEN RECEPTOR-MODIFIED T CELL AND USE THEREOF. Applicant: PERSONGEN BIOTHERAPEUTICS (SUZHOU) CO., LTD. The sequence listing filed with the application follows.

SEQUENCE LISTING (19 sequences)

SEQ ID NO: 1 - protein, 120 aa, Artificial Sequence
  Murine VH
EVTLVESGGGLVKPGGSLKLSCAASGFTFSTYVMSWVRQTPEKRLEWVASILSGGTSFYADNVKGRFTISRENARNILYLQMSSLKSEDTAMYYCVRRYGHDHYYAMDYWGQGTSVTVSS

SEQ ID NO: 2 - protein, 7 aa, Artificial Sequence
  VH CDR1
GFTFSTY

SEQ ID NO: 3 - protein, 5 aa, Artificial Sequence
  VH CDR2
LSGGT

SEQ ID NO: 4 - protein, 12 aa, Artificial Sequence
  VH CDR3
RYGHDHYYAMDY

SEQ ID NO: 5 - protein, 108 aa, Artificial Sequence
  Murine VL
QIVLTQSPANMSASLGERVTMTCAASSSVSSSYLHWYQQKPGSSPKLWIYSTSNLASGVPGRFNGSGSGTSYSLTISSMEAEDAATYYCHQYHRSPWTFGGGTKLEIK

SEQ ID NO: 6 - protein, 12 aa, Artificial Sequence
  VL CDR1
AASSSVSSSYLH

SEQ ID NO: 7 - protein, 7 aa, Artificial Sequence
  VL CDR2
STSNLAS

SEQ ID NO: 8 - protein, 8 aa, Artificial Sequence
  VL CDR3
QYHRSPWT

SEQ ID NO: 9 - protein, 120 aa, Artificial Sequence
  Humanized VH (T1H1)
EVQLVESGGGLIQPGGSLRLSCAASGFTFSTYVMSWVRQAPGKGLEWVSSILSGGTSFYADNVKGRFTISRDNSKNTLYLQMNSLRAEDTAVYYCARRYGHDHYYAMDYWGQGTLVTVSS

SEQ ID NO: 10 - protein, 108 aa, Artificial Sequence
  Humanized VL (T1L1)
EIVLTQSPATLSLSPGERATLSCAASSSVSSSYLHWYQQKPGLAPRLLIYSTSNLASGIPDRFSGSGSGTDFTLTISRLEPEDFAVYYCQQYHRSPWTFGGGTKVEIK

SEQ ID NO: 11 - protein, 120 aa, Artificial Sequence
  Humanized VH (T2H1)
EVQLVESGGGVVRPGGSLRLSCAASGFTFSTYVMSWVRQAPGKGLEWVSSILSGGTSFYADNVKGRFTISRDNAKNSLYLQMNSLRAEDTALYHCARRYGHDHYYAMDYWGQGTTVTVSS

SEQ ID NO: 12 - protein, 108 aa, Artificial Sequence
  Humanized VH (T2L1)
DIQMTQSPSTLSASVGDRVTITCAASSSVSSSYLHWYQQKPGKAPKLLIYSTSNLASGVPSRFSGSGSGTEFTLTISSLQPDDFATYYCQQYHRSPWTFGQGTKLEIK

SEQ ID NO: 13 - protein, 248 aa, Artificial Sequence
  Humanized scFv (T1H1-T1L1)
EVQLVESGGGLIQPGGSLRLSCAASGFTFSTYVMSWVRQAPGKGLEWVSSILSGGTSFYADNVKGRFTISRDNSKNTLYLQMNSLRAEDTAVYYCARRYGHDHYYAMDYWGQGTLVTVSSGGGGSGGGGSGGGGSGGGGSEIVLTQSPATLSLSPGERATLSCAASSSVSSSYLHWYQQKPGLAPRLLIYSTSNLASGIPDRFSGSGSGTDFTLTISRLEPEDFAVYYCQQYHRSPWTFGGGTKVEIK

SEQ ID NO: 14 - protein, 248 aa, Artificial Sequence
  Humanized scFv (T2H1-T2L1)
EVQLVESGGGVVRPGGSLRLSCAASGFTFSTYVMSWVRQAPGKGLEWVSSILSGGTSFYADNVKGRFTISRDNAKNSLYLQMNSLRAEDTALYHCARRYGHDHYYAMDYWGQGTTVTVSSGGGGSGGGGSGGGGSGGGGSDIQMTQSPSTLSASVGDRVTITCAASSSVSSSYLHWYQQKPGKAPKLLIYSTSNLASGVPSRFSGSGSGTEFTLTISSLQPDDFATYYCQQYHRSPWTFGQGTKLEIK

SEQ ID NO: 15 - protein, 335 aa, Artificial Sequence
  tEGFR
RKVCNGIGIGEFKDSLSINATNIKHFKNCTSISGDLHILPVAFRGDSFTHTPPLDPQELDILKTVKEITGFLLIQAWPENRTDLHAFENLEIIRGRTKQHGQFSLAVVSLNITSLGLRSLKEISDGDVIISGNKNLCYANTINWKKLFGTSGQKTKIISNRGENSCKATGQVCHALCSPEGCWGPEPRDCVSCRNVSRGRECVDKCNLLEGEPREFVENSECIQCHPECLPQAMNITCTGRGPDNCIQCAHYIDGPHCVKTCPAGVMGENNTLVWKYADAGHVCHLCHPNCTYGCTGPGLEGCPTNGPKIPSIATGMVGALLLLLVVALGIGLFM

SEQ ID NO: 16 - protein, 492 aa, Artificial Sequence
  alpha hB7-H3 CAR
MALPVTALLLPLALLLHAARPEVQLVESGGGLIQPGGSLRLSCAASGFTFSTYVMSWVRQAPGKGLEWVSSILSGGTSFYADNVKGRFTISRDNSKNTLYLQMNSLRAEDTAVYYCARRYGHDHYYAMDYWGQGTLVTVSSGGGGSGGGGSGGGGSGGGGSEIVLTQSPATLSLSPGERATLSCAASSSVSSSYLHWYQQKPGLAPRLLIYSTSNLASGIPDRFSGSGSGTDFTLTISRLEPEDFAVYYCQQYHRSPWTFGGGTKVEIKTTTPAPRPPTPAPTIASQPLSLRPEACRPAAGGAVHTRGLDFACDIYIWAPLAGTCGVLLLSLVITLYCKRGRKKLLYIFKQPFMRPVQTTQEEDGCSCRFPEEEEGGCELRVKFSRSADAPAYKQGQNQLYNELNLGRREEYDVLDKRRGRDPEMGGKPRRKNPQEGLYNELQKDKMAEAYSEIGMKGERRRGKGHDGLYQGLSTATKDTYDALHMQALPPR

SEQ ID NO: 17 - protein, 5 aa, Artificial Sequence
  Linker
GGGGS

SEQ ID NO: 18 - protein, 248 aa, Artificial Sequence
  Murine scFv (mB7-H3)
EVTLVESGGGLVKPGGSLKLSCAASGFTFSTYVMSWVRQTPEKRLEWVASILSGGTSFYADNVKGRFTISRENARNILYLQMSSLKSEDTAMYYCVRRYGHDHYYAMDYWGQGTSVTVSSGGGGSGGGGSGGGGSGGGGSQIVLTQSPANMSASLGERVTMTCAASSSVSSSYLHWYQQKPGSSPKLWIYSTSNLASGVPGRFNGSGSGTSYSLTISSMEAEDAATYYCHQYHRSPWTFGGGTKLEIK

SEQ ID NO: 19 - protein, 710 aa, Artificial Sequence
  Third-generation B7-H3-CAR
MALPVTALLLPLALLLHAARPEVQLVESGGGLIQPGGSLRLSCAASGFTFSTYVMSWVRQAPGKGLEWVSSILSGGTSFYADNVKGRFTISRDNSKNTLYLQMNSLRAEDTAVYYCARRYGHDHYYAMDYWGQGTLVTVSSGGGGSGGGGSGGGGSGGGGSEIVLTQSPATLSLSPGERATLSCAASSSVSSSYLHWYQQKPGLAPRLLIYSTSNLASGIPDRFSGSGSGTDFTLTISRLEPEDFAVYYCQQYHRSPWTFGGGTKVEIKESKYGPPCPPCPAPEFEGGPSVFLFPPKPKDTLMISRTPEVTCVVVDVSQEDPEVQFNWYVDGVEVHNAKTKPREEQFQSTYRVVSVLTVLHQDWLNGKEYKCKVSNKGLPSSIEKTISKAKGQPREPQVYTLPPSQEEMTKNQVSLTCLVKGFYPSDIAVEWESNGQPENNYKTTPPVLDSDGSFFLYSRLTVDKSRWQEGNVFSCSVMHEALHNHYTQKSLSLSLGKWLPIGCAAFVVVCILGCILICWLTKKKYSSSVHDPNGEYMFMRAVNTAKKSRLTDVTLKRGRKKLLYIFKQPFMRPVQTTQEEDGCSCRFPEEEEGGCELRVKFSRSADAPAYKQGQNQLYNELNLGRREEYDVLDKRRGRDPEMGGKPRRKNPQEGLYNELQKDKMAEAYSEIGMKGERRRGKGHDGLYQGLSTATKDTYDALHMQALPPR